European Patent Application EP 4 379 055 A1, published June 5, 2024. Title: 단백질 발현을 위한 mRNA와 이를 위한 주형. Applicant: 에스케이바이오사이언스(주). The sequence listing filed with the application follows.

SEQUENCE LISTING (23 sequences)

SEQ ID NO: 1 - DNA, 37 bp, synthetic construct
  source 1..37: mol_type = other DNA
actcttctggtccccacagactcagagagaagccacc

SEQ ID NO: 2 - DNA, 114 bp, synthetic construct
  source 1..114: mol_type = other DNA
caatttctattaaaggttcctttgttccctaagtccaactactaaactgggggatattatgaagggccttgagcatctggattctgcctaataaaaaacatttattttcattgc

SEQ ID NO: 3 - DNA, 270 bp, synthetic construct
  source 1..270: mol_type = other DNA
agctcgcttgtcaatttctattaaaggttcctttgttccctaagtccaactactaaactgggggatattatgaagggccttgagcatctggattctgcctaataaaaaacatttattttcattgcatcgatagctcgctttcttgctgtccaatttctattaaaggttcctttgttccctaagtccaactactaaactgggggatattatgaagggccttgagcatctggattctgcctaataaaaaacatttattttcattgcccgcgg

SEQ ID NO: 4 - DNA, 23 bp, synthetic construct
  source 1..23: mol_type = other DNA
taatacgactcactatagggaga

SEQ ID NO: 5 - DNA, 112 bp, synthetic construct
  source 1..112: mol_type = other DNA
aaaaaaaaaaaaaaaaaaaaaaaaaaaaaagcatatgactaaaaaaaaaaaaaaaaaaaaaaaaaaaaaaaaaaaaaaaaaaaaaaaaaaaaaaaaaaaaaaaaaaaaaaaa

SEQ ID NO: 6 - DNA, 72 bp, synthetic construct
  source 1..72: mol_type = other DNA
ggtacctaatacgactcactatagggagaactcttctggtccccacagactcagagagaagccaccggatcc

SEQ ID NO: 7 - DNA, 406 bp, synthetic construct
  source 1..406: mol_type = other DNA
tctagaagctcgcttgtcaatttctattaaaggttcctttgttccctaagtccaactactaaactgggggatattatgaagggccttgagcatctggattctgcctaataaaaaacatttattttcattgcatcgatagctcgctttcttgctgtccaatttctattaaaggttcctttgttccctaagtccaactactaaactgggggatattatgaagggccttgagcatctggattctgcctaataaaaaacatttattttcattgcccgcggaaaaaaaaaaaaaaaaaaaaaaaaaaaaaagcatatgactaaaaaaaaaaaaaaaaaaaaaaaaaaaaaaaaaaaaaaaaaaaaaaaaaaaaaaaaaaaaaaaaaaaaaaaagtcttcgatatcaagctt

SEQ ID NO: 8 - DNA, 3119 bp, synthetic construct
  source 1..3119: mol_type = other DNA
tcgcgcgtttcggtgatgacggtgaaaacctctgacacatgcagctcccggagacggtcacagcttgtctgtaagcggatgccgggagcagacaagcccgtcagggcgcgtcagcgggtgttggcgggtgtcggggctggcttaactatgcggcatcagagcagattgtactgagagtgcaccatatgcggtgtgaaataccgcacagatgcgtaaggagaaaataccgcatcaggcgccattcgccattcaggctgcgcaactgttgggaagggcgatcggtgcgggcctcttcgctattacgccagctggcgaaagggggatgtgctgcaaggcgattaagttgggtaacgccagggttttcccagtcacgacgttgtaaaacgacggccagtgaattcgagctcggtacctaatacgactcactatagggagaactcttctggtccccacagactcagagagaagccaccggatcctctagaagctcgcttgtcaatttctattaaaggttcctttgttccctaagtccaactactaaactgggggatattatgaagggccttgagcatctggattctgcctaataaaaaacatttattttcattgcatcgatagctcgctttcttgctgtccaatttctattaaaggttcctttgttccctaagtccaactactaaactgggggatattatgaagggccttgagcatctggattctgcctaataaaaaacatttattttcattgcccgcggaaaaaaaaaaaaaaaaaaaaaaaaaaaaaagcatatgactaaaaaaaaaaaaaaaaaaaaaaaaaaaaaaaaaaaaaaaaaaaaaaaaaaaaaaaaaaaaaaaaaaaaaaaagtcttcgatatcaagcttggcgtaatcatggtcatagctgtttcctgtgtgaaattgttatccgctcacaattccacacaacatacgagccggaagcataaagtgtaaagcctggggtgcctaatgagtgagctaactcacattaattgcgttgcgctcactgcccgctttccagtcgggaaacctgtcgtgccagctgcattaatgaatcggccaacgcgcggggagaggcggtttgcgtattgggcgctcttccgcttcctcgctcactgactcgctgcgctcggtcgttcggctgcggcgagcggtatcagctcactcaaaggcggtaatacggttatccacagaatcaggggataacgcaggaaagaacatgtgagcaaaaggccagcaaaaggccaggaaccgtaaaaaggccgcgttgctggcgtttttccataggctccgcccccctgacgagcatcacaaaaatcgacgctcaagtcagaggtggcgaaacccgacaggactataaagataccaggcgtttccccctggaagctccctcgtgcgctctcctgttccgaccctgccgcttaccggatacctgtccgcctttctcccttcgggaagcgtggcgctttctcatagctcacgctgtaggtatctcagttcggtgtaggtcgttcgctccaagctgggctgtgtgcacgaaccccccgttcagcccgaccgctgcgccttatccggtaactatcgtcttgagtccaacccggtaagacacgacttatcgccactggcagcagccactggtaacaggattagcagagcgaggtatgtaggcggtgctacagagttcttgaagtggtggcctaactacggctacactagaagaacagtatttggtatctgcgctctgctgaagccagttaccttcggaaaaagagttggtagctcttgatccggcaaacaaaccaccgctggtagcggtggtttttttgtttgcaagcagcagattacgcgcagaaaaaaaggatctcaagaagatcctttgatcttttctacggggtctgacgctcagtggaacgaaaactcacgttaagggattttggtcatgagattatcaaaaaggatcttcacctagatccttttaaattaaaaatgaagttttaaatcaatctaaagtatatatgagtaaacttggtctgacagttaccaatgcttaatcagtgaggcacctatctcagcgatctgtctatttcgttcatccatagttgcctgactccccgtcgtgtagataactacgatacgggagggcttaccatctggccccagtgctgcaatgataccgcgagacccacgctcaccggctccagatttatcagcaataaaccagccagccggaagggccgagcgcagaagtggtcctgcaactttatccgcctccatccagtctattaattgttgccgggaagctagagtaagtagttcgccagttaatagtttgcgcaacgttgttgccattgctacaggcatcgtggtgtcacgctcgtcgtttggtatggcttcattcagctccggttcccaacgatcaaggcgagttacatgatcccccatgttgtgcaaaaaagcggttagctccttcggtcctccgatcgttgtcagaagtaagttggccgcagtgttatcactcatggttatggcagcactgcataattctcttactgtcatgccatccgtaagatgcttttctgtgactggtgagtactcaaccaagtcattctgagaatagtgtatgcggcgaccgagttgctcttgcccggcgtcaatacgggataataccgcgccacatagcagaactttaaaagtgctcatcattggaaaacgttcttcggggcgaaaactctcaaggatcttaccgctgttgagatccagttcgatgtaacccactcgtgcacccaactgatcttcagcatcttttactttcaccagcgtttctgggtgagcaaaaacaggaaggcaaaatgccgcaaaaaagggaataagggcgacacggaaatgttgaatactcatactcttcctttttcaatattattgaagcatttatcagggttattgtctcatgagcggatacatatttgaatgtatttagaaaaataaacaaataggggttccgcgcacatttccccgaaaagtgccacctgacgtctaagaaaccattattatcatgacattaacctataaaaataggcgtatcacgaggccctttcgtc

SEQ ID NO: 9 - DNA, 955 bp, synthetic construct
  source 1..955: mol_type = other DNA
ggatccgaccatgacttcgaaagtttatgatccagaacaaaggaaacggatgataactggtccgcagtggtgggccagatgtaaacaaatgaatgttcttgattcatttattaattattatgattcagaaaaacatgcagaaaatgctgttatttttttacatggtaacgcggcctcttcttatttatggcgacatgttgtgccacatattgagccagtagcgcggtgtattataccagaccttattggtatgggcaaatcaggcaaatctggtaatggttcttataggttacttgatcattacaaatatcttactgcatggtttgaacttcttaatttaccaaagaagatcatttttgtcggccatgattggggtgcttgtttggcatttcattatagccatgagcatcaagataagatcaaagcaatagttcacgctgaaagtgtagtagatgtgattgaatcatgggatgaatggcctgatattgaagaagatattgcgttgatcaaatctgaagaaggagaaaaaatggttttggagaataacttcttcgtggaaaccatgttgccatcaaaaatcatgagaaagttagaaccagaagaatttgcagcatatcttgaaccattcaaagagaaaggtgaagttcgtcgtccaacattatcatggcctcgtgaaatcccgttagtaaaaggtggtaaacctgacgttgtacaaattgttaggaattataatgcttatctacgtgcaagtgatgatttaccaaaaatgtttattgaatcggacccaggattcttttccaatgctattgttgaaggtgccaagaagtttcctaatactgaatttgtcaaagtaaaaggtcttcatttttcgcaagaagatgcacctgatgaaatgggaaaatatatcaaatcgttcgttgagcgagttctcaaaaatgaacaataatagtctaga

SEQ ID NO: 10 - DNA, 4061 bp, synthetic construct
  source 1..4061: mol_type = other DNA
tcgcgcgtttcggtgatgacggtgaaaacctctgacacatgcagctcccggagacggtcacagcttgtctgtaagcggatgccgggagcagacaagcccgtcagggcgcgtcagcgggtgttggcgggtgtcggggctggcttaactatgcggcatcagagcagattgtactgagagtgcaccatatgcggtgtgaaataccgcacagatgcgtaaggagaaaataccgcatcaggcgccattcgccattcaggctgcgcaactgttgggaagggcgatcggtgcgggcctcttcgctattacgccagctggcgaaagggggatgtgctgcaaggcgattaagttgggtaacgccagggttttcccagtcacgacgttgtaaaacgacggccagtgaattcgagctcggtacctaatacgactcactatagggagaactcttctggtccccacagactcagagagaagccaccggatccgaccatgacttcgaaagtttatgatccagaacaaaggaaacggatgataactggtccgcagtggtgggccagatgtaaacaaatgaatgttcttgattcatttattaattattatgattcagaaaaacatgcagaaaatgctgttatttttttacatggtaacgcggcctcttcttatttatggcgacatgttgtgccacatattgagccagtagcgcggtgtattataccagaccttattggtatgggcaaatcaggcaaatctggtaatggttcttataggttacttgatcattacaaatatcttactgcatggtttgaacttcttaatttaccaaagaagatcatttttgtcggccatgattggggtgcttgtttggcatttcattatagccatgagcatcaagataagatcaaagcaatagttcacgctgaaagtgtagtagatgtgattgaatcatgggatgaatggcctgatattgaagaagatattgcgttgatcaaatctgaagaaggagaaaaaatggttttggagaataacttcttcgtggaaaccatgttgccatcaaaaatcatgagaaagttagaaccagaagaatttgcagcatatcttgaaccattcaaagagaaaggtgaagttcgtcgtccaacattatcatggcctcgtgaaatcccgttagtaaaaggtggtaaacctgacgttgtacaaattgttaggaattataatgcttatctacgtgcaagtgatgatttaccaaaaatgtttattgaatcggacccaggattcttttccaatgctattgttgaaggtgccaagaagtttcctaatactgaatttgtcaaagtaaaaggtcttcatttttcgcaagaagatgcacctgatgaaatgggaaaatatatcaaatcgttcgttgagcgagttctcaaaaatgaacaataatagtctagaagctcgcttgtcaatttctattaaaggttcctttgttccctaagtccaactactaaactgggggatattatgaagggccttgagcatctggattctgcctaataaaaaacatttattttcattgcatcgatagctcgctttcttgctgtccaatttctattaaaggttcctttgttccctaagtccaactactaaactgggggatattatgaagggccttgagcatctggattctgcctaataaaaaacatttattttcattgcccgcggaaaaaaaaaaaaaaaaaaaaaaaaaaaaaagcatatgactaaaaaaaaaaaaaaaaaaaaaaaaaaaaaaaaaaaaaaaaaaaaaaaaaaaaaaaaaaaaaaaaaaaaaaaagtcttcgatatcaagctggcgtaatcatggtcatagctgtttcctgtgtgaaattgttatccgctcacaattccacacaacatacgagccggaagcataaagtgtaaagcctggggtgcctaatgagtgagctaactcacattaattgcgttgcgctcactgcccgctttccagtcgggaaacctgtcgtgccagctgcattaatgaatcggccaacgcgcggggagaggcggtttgcgtattgggcgctcttccgcttcctcgctcactgactcgctgcgctcggtcgttcggctgcggcgagcggtatcagctcactcaaaggcggtaatacggttatccacagaatcaggggataacgcaggaaagaacatgtgagcaaaaggccagcaaaaggccaggaaccgtaaaaaggccgcgttgctggcgtttttccataggctccgcccccctgacgagcatcacaaaaatcgacgctcaagtcagaggtggcgaaacccgacaggactataaagataccaggcgtttccccctggaagctccctcgtgcgctctcctgttccgaccctgccgcttaccggatacctgtccgcctttctcccttcgggaagcgtggcgctttctcatagctcacgctgtaggtatctcagttcggtgtaggtcgttcgctccaagctgggctgtgtgcacgaaccccccgttcagcccgaccgctgcgccttatccggtaactatcgtcttgagtccaacccggtaagacacgacttatcgccactggcagcagccactggtaacaggattagcagagcgaggtatgtaggcggtgctacagagttcttgaagtggtggcctaactacggctacactagaagaacagtatttggtatctgcgctctgctgaagccagttaccttcggaaaaagagttggtagctcttgatccggcaaacaaaccaccgctggtagcggtggtttttttgtttgcaagcagcagattacgcgcagaaaaaaaggatctcaagaagatcctttgatcttttctacggggtctgacgctcagtggaacgaaaactcacgttaagggattttggtcatgagattatcaaaaaggatcttcacctagatccttttaaattaaaaatgaagttttaaatcaatctaaagtatatatgagtaaacttggtctgacagttaccaatgcttaatcagtgaggcacctatctcagcgatctgtctatttcgttcatccatagttgcctgactccccgtcgtgtagataactacgatacgggagggcttaccatctggccccagtgctgcaatgataccgcgagacccacgctcaccggctccagatttatcagcaataaaccagccagccggaagggccgagcgcagaagtggtcctgcaactttatccgcctccatccagtctattaattgttgccgggaagctagagtaagtagttcgccagttaatagtttgcgcaacgttgttgccattgctacaggcatcgtggtgtcacgctcgtcgtttggtatggcttcattcagctccggttcccaacgatcaaggcgagttacatgatcccccatgttgtgcaaaaaagcggttagctccttcggtcctccgatcgttgtcagaagtaagttggccgcagtgttatcactcatggttatggcagcactgcataattctcttactgtcatgccatccgtaagatgcttttctgtgactggtgagtactcaaccaagtcattctgagaatagtgtatgcggcgaccgagttgctcttgcccggcgtcaatacgggataataccgcgccacatagcagaactttaaaagtgctcatcattggaaaacgttcttcggggcgaaaactctcaaggatcttaccgctgttgagatccagttcgatgtaacccactcgtgcacccaactgatcttcagcatcttttactttcaccagcgtttctgggtgagcaaaaacaggaaggcaaaatgccgcaaaaaagggaataagggcgacacggaaatgttgaatactcatactcttcctttttcaatattattgaagcatttatcagggttattgtctcatgagcggatacatatttgaatgtatttagaaaaataaacaaataggggttccgcgcacatttccccgaaaagtgccacctgacgtctaagaaaccattattatcatgacattaacctataaaaataggcgtatcacgaggccctttcgtc

SEQ ID NO: 11 - DNA, 88 bp, synthetic construct
  source 1..88: mol_type = other DNA
ggtacctaatacgactcactatagggggaaataagagagaaaagaagagtaagaagaaatataagaccccggcgccgccaccggatcc

SEQ ID NO: 12 - DNA, 123 bp, synthetic construct
  source 1..123: mol_type = other DNA
tctagagctggagcctcggtggcctagcttcttgccccttgggcctccccccagcccctcctccccttcctgcacccgtacccccgtggtctttgaataaagtctgagtgggcggcaccgcgg

SEQ ID NO: 13 - DNA, 85 bp, synthetic construct
  source 1..85: mol_type = other DNA
ggtacctaatacgactcactatagggagaataaactagtattcttctggtccccacagactcagagagaacccgccaccggatcc

SEQ ID NO: 14 - DNA, 307 bp, synthetic construct
  source 1..307: mol_type = other DNA
tctagactcgagctggtactgcatgcacgcaatgctagctgcccctttcccgtcctgggtaccccgagtctcccccgacctcgggtcccaggtatgctcccacctccacctgccccactcaccacctctgctagttccagacacctcccaagcacgcagcaatgcagctcaaaacgcttagcctagccacacccccacgggaaacagcagtgattaacctttagcaataaacgaaagtttaactaagctatactaaccccagggttggtcaatttcgtgccagccacaccctggagctagcccgcgg

SEQ ID NO: 15 - DNA, 23 bp, synthetic construct
  source 1..23: mol_type = other DNA
taatacgactcactataaggaga

SEQ ID NO: 16 - DNA, 72 bp, synthetic construct
  source 1..72: mol_type = other DNA
ggtacctaatacgactcactataaggagaactcttctggtccccacagactcagagagaagccaccggatcc

SEQ ID NO: 17 - DNA, 316 bp, synthetic construct
  source 1..316: mol_type = other DNA
tctagaagctcgcttgtcaatttctattaaaggttcctttgttccctaagtccaactactaaactgggggatattatgaagggccttgagcatctggattctgcctaataaaaaacatttattttcattgcatcgatagctcgctttcttgctgtccaatttctattaaaggttcctttgttccctaagtccaactactaaactgggggatattatgaagggccttgagcatctggattctgcctaataaaaaacatttattttcattgcccgcggaaaaaaaaaaaaaaaaaaaaaagtcttcgatatcaagctt

SEQ ID NO: 18 - DNA, 3029 bp, synthetic construct
  source 1..3029: mol_type = other DNA
tcgcgcgtttcggtgatgacggtgaaaacctctgacacatgcagctcccggagacggtcacagcttgtctgtaagcggatgccgggagcagacaagcccgtcagggcgcgtcagcgggtgttggcgggtgtcggggctggcttaactatgcggcatcagagcagattgtactgagagtgcaccatatgcggtgtgaaataccgcacagatgcgtaaggagaaaataccgcatcaggcgccattcgccattcaggctgcgcaactgttgggaagggcgatcggtgcgggcctcttcgctattacgccagctggcgaaagggggatgtgctgcaaggcgattaagttgggtaacgccagggttttcccagtcacgacgttgtaaaacgacggccagtgaattcgagctcggtacctaatacgactcactataaggagaactcttctggtccccacagactcagagagaagccaccggatcctctagaagctcgcttgtcaatttctattaaaggttcctttgttccctaagtccaactactaaactgggggatattatgaagggccttgagcatctggattctgcctaataaaaaacatttattttcattgcatcgatagctcgctttcttgctgtccaatttctattaaaggttcctttgttccctaagtccaactactaaactgggggatattatgaagggccttgagcatctggattctgcctaataaaaaacatttattttcattgcccgcggaaaaaaaaaaaaaaaaaaaaaagtcttcgatatcaagcttggcgtaatcatggtcatagctgtttcctgtgtgaaattgttatccgctcacaattccacacaacatacgagccggaagcataaagtgtaaagcctggggtgcctaatgagtgagctaactcacattaattgcgttgcgctcactgcccgctttccagtcgggaaacctgtcgtgccagctgcattaatgaatcggccaacgcgcggggagaggcggtttgcgtattgggcgctcttccgcttcctcgctcactgactcgctgcgctcggtcgttcggctgcggcgagcggtatcagctcactcaaaggcggtaatacggttatccacagaatcaggggataacgcaggaaagaacatgtgagcaaaaggccagcaaaaggccaggaaccgtaaaaaggccgcgttgctggcgtttttccataggctccgcccccctgacgagcatcacaaaaatcgacgctcaagtcagaggtggcgaaacccgacaggactataaagataccaggcgtttccccctggaagctccctcgtgcgctctcctgttccgaccctgccgcttaccggatacctgtccgcctttctcccttcgggaagcgtggcgctttctcatagctcacgctgtaggtatctcagttcggtgtaggtcgttcgctccaagctgggctgtgtgcacgaaccccccgttcagcccgaccgctgcgccttatccggtaactatcgtcttgagtccaacccggtaagacacgacttatcgccactggcagcagccactggtaacaggattagcagagcgaggtatgtaggcggtgctacagagttcttgaagtggtggcctaactacggctacactagaagaacagtatttggtatctgcgctctgctgaagccagttaccttcggaaaaagagttggtagctcttgatccggcaaacaaaccaccgctggtagcggtggtttttttgtttgcaagcagcagattacgcgcagaaaaaaaggatctcaagaagatcctttgatcttttctacggggtctgacgctcagtggaacgaaaactcacgttaagggattttggtcatgagattatcaaaaaggatcttcacctagatccttttaaattaaaaatgaagttttaaatcaatctaaagtatatatgagtaaacttggtctgacagttaccaatgcttaatcagtgaggcacctatctcagcgatctgtctatttcgttcatccatagttgcctgactccccgtcgtgtagataactacgatacgggagggcttaccatctggccccagtgctgcaatgataccgcgagacccacgctcaccggctccagatttatcagcaataaaccagccagccggaagggccgagcgcagaagtggtcctgcaactttatccgcctccatccagtctattaattgttgccgggaagctagagtaagtagttcgccagttaatagtttgcgcaacgttgttgccattgctacaggcatcgtggtgtcacgctcgtcgtttggtatggcttcattcagctccggttcccaacgatcaaggcgagttacatgatcccccatgttgtgcaaaaaagcggttagctccttcggtcctccgatcgttgtcagaagtaagttggccgcagtgttatcactcatggttatggcagcactgcataattctcttactgtcatgccatccgtaagatgcttttctgtgactggtgagtactcaaccaagtcattctgagaatagtgtatgcggcgaccgagttgctcttgcccggcgtcaatacgggataataccgcgccacatagcagaactttaaaagtgctcatcattggaaaacgttcttcggggcgaaaactctcaaggatcttaccgctgttgagatccagttcgatgtaacccactcgtgcacccaactgatcttcagcatcttttactttcaccagcgtttctgggtgagcaaaaacaggaaggcaaaatgccgcaaaaaagggaataagggcgacacggaaatgttgaatactcatactcttcctttttcaatattattgaagcatttatcagggttattgtctcatgagcggatacatatttgaatgtatttagaaaaataaacaaataggggttccgcgcacatttccccgaaaagtgccacctgacgtctaagaaaccattattatcatgacattaacctataaaaataggcgtatcacgaggccctttcgtc

SEQ ID NO: 19 - DNA, 3831 bp, synthetic construct
  source 1..3831: mol_type = other DNA
ggatccaccatgttcgtgttcctggtgctgctgcctctggtgtccagccagtgcgtgaattttaccactcggacccagttaccgcctgcttataccaacagcttcaccagaggagtgtactatcctgacaaggtgttcagaagctccgtgctccacagcacacaggacctgtttctgccattcttcagcaatgtgacctggttccacgccatccacgtgtccggaaccaacggcacaaagagatttgctaaccctgttctgccattcaacgacggcgtgtacttcgcttccacagagaagtccaacatcatcagaggctggatcttcggcaccaccctggatagcaagacccagagcctcctgatcgtgaacaacgccacgaacgtcgtgatcaaggtgtgcgagttccagttctgtaatgaccccttcttgggcgtttattaccacaagaacaacaagagctggatggaatctgagtttagagtatattccagcgctaacaattgcaccttcgagtacgttagccagcccttcctcatggacctggaaggcaagcagggcaatttcaagaacctgagagagttcgtattcaagaacatcgacggctacttcaagatctacagcaagcacacacctatcaacctagtgcgcgggctgccacagggcttcagcgctctggaacccctggtcgatctgcctataggcatcaacatcaccagattccaaaccctgcacatctcctacctgacccctggagacagctctagcggatggaccgccggcgctgccgcctactacgtaggctacctgcagcctaggaccttcctgctgaagtacaacgagaacggcaccatcaccgatgccgtggactgtgccctggaccctctatctgagacaaagtgcaccctgaagagcttcaccgtggaaaagggcatctaccagaccagtaactttagagtgcagcccaccgaaagcatcgtgagattccctaacatcaccaatctgtgtcctttcggcgaggtgtttaacgccacaagattcgccagcgtctacgcctggaaccggaagcggatcagcaactgcgtggctgattactccgtcctttataacagcgctagcttcagcacatttaaatgctacggagtgagcccaacaaagctgaacgacctgtgcttcaccaacgtgtacgccgatagcttcgtgatcagaggcgatgaggtgagacagattgcccctggccagacaggcaacatcgccgattacaactataagctgcccgacgacttcaccggctgtgtgatcgcttggaacagcaacaacctcgatagcaaggtgggaggaaattacaactacctgtataggctgttcagaaaaagcaatctgaagcctttcgagagagacatcagcaccgaaatctaccaggccggatctacaccttgcaacggcgtgaagggcttcaactgttacttccctctgcaatcatacggcttccagcctacctacggcgtgggctaccagccctaccgagtcgtggtgctgagctttgaactgctgcatgcgcccgcgacagtgtgcggccctaagaaaagcaccaacctggtgaagaacaaatgcgtgaacttcaactttaacgggctgactggcaccggtgtcctgaccgagagcaacaagaagtttctgcccttccagcaattcggcagagacatcgccgacaccaccgacgccgtccgcgacccccagaccctggagatcctcgatattacaccttgtagcttcggcggcgtcagcgttatcacacccggaacaaacacaagcaatcaggtggccgtgctgtaccagggcgtgaactgcacagaggtgcctgtggcaatccacgccgaccagctgacccctacctggcgggtgtactctaccggcagcaatgtgttccagacaagagccggctgcctgatcggcgccgaacacgtgaacaacagctacgaatgtgacatccctattggcgccggaatctgcgcctcttaccagacacagaccaactcacctcggagagccagatctgtggcgagccaatctatcatcgcctacaccatgtctctcggcgtggaaaactctgtggcctacagcaacaactctatcgcaatccccacaaacttcaccatcagcgtgacaaccgagatcctgccggtgtctatgaccaagacatccgtggactgcaccatgtacatctgcggcgactccacagaatgcagcaatctgctgttgcagtacggcagcttctgcacacaattaaatcgtgccctgacaggcattgccgtggaacaggataagaatacccaggaagtgttcgcccaggtgaagcagatttacaagaccccacctatcaaggacttcggcggctttaatttctcccagatcctgcctgacccctctaagccttctaagagaagttttatcgaggacctgctgttcaataaagtgaccctggccgatgccgggttcatcaagcagtacggcgattgcctgggcgacatcgccgccagagatcttatttgcgcccagaaattcaacggactgacagtgctgcctcctttgctgaccgacgagatgattgcccagtataccagcgccctgctggccggaaccatcacgtccggctggacattcggcgccggcgccgccttgcagatccccttcgccatgcagatggcctaccggtttaatggcatcggcgtgacgcagaacgtgctgtacgagaaccagaaactgatcgctaaccagtttaactccgccatcggcaagatccaggacagcctgagctccaccgccagcgccctgggcaagctgcaagacgtggtgaaccagaatgcccaagccctgaacaccctggtgaagcagctgagctctaacttcggcgccatcagcagcgtgctgaacgacattctgagcagactggaccctccagaagccgaggtgcagatcgaccggctgatcaccggccggctgcaatccctgcagacctacgtgacccaacagctgatccgggccgccgagatcagagcctcggctaacctggccgccacaaagatgagcgagtgcgtgctgggccagtctaaaagagtggacttctgcggtaaaggataccacctgatgagttttcctcaaagcgcccctcacggcgtggtgttcctgcatgtgacatacgtccccgcccaggagaagaattttaccacagcccctgctatctgtcacgatggcaaagcccacttcccacgggagggcgtgtttgtgagcaacggcacccactggttcgtgacccagagaaacttctacgaacctcagatcatcacgaccgacaacacctttgtgagcggcaactgcgacgtggtgatcggcatcgtgaacaataccgtgtacgaccctctgcagcccgaactggattctttcaaggaggaactggacaagtacttcaagaaccacaccagccctgatgtggacctgggcgacatcagcggcatcaatgcctccgtggtgaatatccagaaagagatcgacagactgaatgaggtggctaagaaccttaatgagagcctgatcgatctgcaggagctgggcaagtacgagcagtacatcaagtggccttggtacatctggctgggattcatcgccggactgatcgctatcgtgatggtcaccatcatgctgtgctgcatgaccagctgctgtagctgcctgaagggatgctgtagctgtggcagctgctgcaagttcgacgaggatgacagcgagcctgtgctgaagggcgtgaagctgcactacacctgataatctaga

SEQ ID NO: 20 - DNA, 6848 bp, synthetic construct
  source 1..6848: mol_type = other DNA
tcgcgcgtttcggtgatgacggtgaaaacctctgacacatgcagctcccggagacggtcacagcttgtctgtaagcggatgccgggagcagacaagcccgtcagggcgcgtcagcgggtgttggcgggtgtcggggctggcttaactatgcggcatcagagcagattgtactgagagtgcaccatatgcggtgtgaaataccgcacagatgcgtaaggagaaaataccgcatcaggcgccattcgccattcaggctgcgcaactgttgggaagggcgatcggtgcgggcctcttcgctattacgccagctggcgaaagggggatgtgctgcaaggcgattaagttgggtaacgccagggttttcccagtcacgacgttgtaaaacgacggccagtgaattcgagctcggtacctaatacgactcactataaggagaactcttctggtccccacagactcagagagaagccaccggatccaccatgttcgtgttcctggtgctgctgcctctggtgtccagccagtgcgtgaattttaccactcggacccagttaccgcctgcttataccaacagcttcaccagaggagtgtactatcctgacaaggtgttcagaagctccgtgctccacagcacacaggacctgtttctgccattcttcagcaatgtgacctggttccacgccatccacgtgtccggaaccaacggcacaaagagatttgctaaccctgttctgccattcaacgacggcgtgtacttcgcttccacagagaagtccaacatcatcagaggctggatcttcggcaccaccctggatagcaagacccagagcctcctgatcgtgaacaacgccacgaacgtcgtgatcaaggtgtgcgagttccagttctgtaatgaccccttcttgggcgtttattaccacaagaacaacaagagctggatggaatctgagtttagagtatattccagcgctaacaattgcaccttcgagtacgttagccagcccttcctcatggacctggaaggcaagcagggcaatttcaagaacctgagagagttcgtattcaagaacatcgacggctacttcaagatctacagcaagcacacacctatcaacctagtgcgcgggctgccacagggcttcagcgctctggaacccctggtcgatctgcctataggcatcaacatcaccagattccaaaccctgcacatctcctacctgacccctggagacagctctagcggatggaccgccggcgctgccgcctactacgtaggctacctgcagcctaggaccttcctgctgaagtacaacgagaacggcaccatcaccgatgccgtggactgtgccctggaccctctatctgagacaaagtgcaccctgaagagcttcaccgtggaaaagggcatctaccagaccagtaactttagagtgcagcccaccgaaagcatcgtgagattccctaacatcaccaatctgtgtcctttcggcgaggtgtttaacgccacaagattcgccagcgtctacgcctggaaccggaagcggatcagcaactgcgtggctgattactccgtcctttataacagcgctagcttcagcacatttaaatgctacggagtgagcccaacaaagctgaacgacctgtgcttcaccaacgtgtacgccgatagcttcgtgatcagaggcgatgaggtgagacagattgcccctggccagacaggcaacatcgccgattacaactataagctgcccgacgacttcaccggctgtgtgatcgcttggaacagcaacaacctcgatagcaaggtgggaggaaattacaactacctgtataggctgttcagaaaaagcaatctgaagcctttcgagagagacatcagcaccgaaatctaccaggccggatctacaccttgcaacggcgtgaagggcttcaactgttacttccctctgcaatcatacggcttccagcctacctacggcgtgggctaccagccctaccgagtcgtggtgctgagctttgaactgctgcatgcgcccgcgacagtgtgcggccctaagaaaagcaccaacctggtgaagaacaaatgcgtgaacttcaactttaacgggctgactggcaccggtgtcctgaccgagagcaacaagaagtttctgcccttccagcaattcggcagagacatcgccgacaccaccgacgccgtccgcgacccccagaccctggagatcctcgatattacaccttgtagcttcggcggcgtcagcgttatcacacccggaacaaacacaagcaatcaggtggccgtgctgtaccagggcgtgaactgcacagaggtgcctgtggcaatccacgccgaccagctgacccctacctggcgggtgtactctaccggcagcaatgtgttccagacaagagccggctgcctgatcggcgccgaacacgtgaacaacagctacgaatgtgacatccctattggcgccggaatctgcgcctcttaccagacacagaccaactcacctcggagagccagatctgtggcgagccaatctatcatcgcctacaccatgtctctcggcgtggaaaactctgtggcctacagcaacaactctatcgcaatccccacaaacttcaccatcagcgtgacaaccgagatcctgccggtgtctatgaccaagacatccgtggactgcaccatgtacatctgcggcgactccacagaatgcagcaatctgctgttgcagtacggcagcttctgcacacaattaaatcgtgccctgacaggcattgccgtggaacaggataagaatacccaggaagtgttcgcccaggtgaagcagatttacaagaccccacctatcaaggacttcggcggctttaatttctcccagatcctgcctgacccctctaagccttctaagagaagttttatcgaggacctgctgttcaataaagtgaccctggccgatgccgggttcatcaagcagtacggcgattgcctgggcgacatcgccgccagagatcttatttgcgcccagaaattcaacggactgacagtgctgcctcctttgctgaccgacgagatgattgcccagtataccagcgccctgctggccggaaccatcacgtccggctggacattcggcgccggcgccgccttgcagatccccttcgccatgcagatggcctaccggtttaatggcatcggcgtgacgcagaacgtgctgtacgagaaccagaaactgatcgctaaccagtttaactccgccatcggcaagatccaggacagcctgagctccaccgccagcgccctgggcaagctgcaagacgtggtgaaccagaatgcccaagccctgaacaccctggtgaagcagctgagctctaacttcggcgccatcagcagcgtgctgaacgacattctgagcagactggaccctccagaagccgaggtgcagatcgaccggctgatcaccggccggctgcaatccctgcagacctacgtgacccaacagctgatccgggccgccgagatcagagcctcggctaacctggccgccacaaagatgagcgagtgcgtgctgggccagtctaaaagagtggacttctgcggtaaaggataccacctgatgagttttcctcaaagcgcccctcacggcgtggtgttcctgcatgtgacatacgtccccgcccaggagaagaattttaccacagcccctgctatctgtcacgatggcaaagcccacttcccacgggagggcgtgtttgtgagcaacggcacccactggttcgtgacccagagaaacttctacgaacctcagatcatcacgaccgacaacacctttgtgagcggcaactgcgacgtggtgatcggcatcgtgaacaataccgtgtacgaccctctgcagcccgaactggattctttcaaggaggaactggacaagtacttcaagaaccacaccagccctgatgtggacctgggcgacatcagcggcatcaatgcctccgtggtgaatatccagaaagagatcgacagactgaatgaggtggctaagaaccttaatgagagcctgatcgatctgcaggagctgggcaagtacgagcagtacatcaagtggccttggtacatctggctgggattcatcgccggactgatcgctatcgtgatggtcaccatcatgctgtgctgcatgaccagctgctgtagctgcctgaagggatgctgtagctgtggcagctgctgcaagttcgacgaggatgacagcgagcctgtgctgaagggcgtgaagctgcactacacctgataatctagaagctcgcttgtcaatttctattaaaggttcctttgttccctaagtccaactactaaactgggggatattatgaagggccttgagcatctggattctgcctaataaaaaacatttattttcattgcatcgatagctcgctttcttgctgtccaatttctattaaaggttcctttgttccctaagtccaactactaaactgggggatattatgaagggccttgagcatctggattctgcctaataaaaaacatttattttcattgcccgcggaaaaaaaaaaaaaaaaaaaaaagtcttcgatatcaagcttggcgtaatcatggtcatagctgtttcctgtgtgaaattgttatccgctcacaattccacacaacatacgagccggaagcataaagtgtaaagcctggggtgcctaatgagtgagctaactcacattaattgcgttgcgctcactgcccgctttccagtcgggaaacctgtcgtgccagctgcattaatgaatcggccaacgcgcggggagaggcggtttgcgtattgggcgctcttccgcttcctcgctcactgactcgctgcgctcggtcgttcggctgcggcgagcggtatcagctcactcaaaggcggtaatacggttatccacagaatcaggggataacgcaggaaagaacatgtgagcaaaaggccagcaaaaggccaggaaccgtaaaaaggccgcgttgctggcgtttttccataggctccgcccccctgacgagcatcacaaaaatcgacgctcaagtcagaggtggcgaaacccgacaggactataaagataccaggcgtttccccctggaagctccctcgtgcgctctcctgttccgaccctgccgcttaccggatacctgtccgcctttctcccttcgggaagcgtggcgctttctcatagctcacgctgtaggtatctcagttcggtgtaggtcgttcgctccaagctgggctgtgtgcacgaaccccccgttcagcccgaccgctgcgccttatccggtaactatcgtcttgagtccaacccggtaagacacgacttatcgccactggcagcagccactggtaacaggattagcagagcgaggtatgtaggcggtgctacagagttcttgaagtggtggcctaactacggctacactagaagaacagtatttggtatctgcgctctgctgaagccagttaccttcggaaaaagagttggtagctcttgatccggcaaacaaaccaccgctggtagcggtggtttttttgtttgcaagcagcagattacgcgcagaaaaaaaggatctcaagaagatcctttgatcttttctacggggtctgacgctcagtggaacgaaaactcacgttaagggattttggtcatgagattatcaaaaaggatcttcacctagatccttttaaattaaaaatgaagttttaaatcaatctaaagtatatatgagtaaacttggtctgacagttaccaatgcttaatcagtgaggcacctatctcagcgatctgtctatttcgttcatccatagttgcctgactccccgtcgtgtagataactacgatacgggagggcttaccatctggccccagtgctgcaatgataccgcgagacccacgctcaccggctccagatttatcagcaataaaccagccagccggaagggccgagcgcagaagtggtcctgcaactttatccgcctccatccagtctattaattgttgccgggaagctagagtaagtagttcgccagttaatagtttgcgcaacgttgttgccattgctacaggcatcgtggtgtcacgctcgtcgtttggtatggcttcattcagctccggttcccaacgatcaaggcgagttacatgatcccccatgttgtgcaaaaaagcggttagctccttcggtcctccgatcgttgtcagaagtaagttggccgcagtgttatcactcatggttatggcagcactgcataattctcttactgtcatgccatccgtaagatgcttttctgtgactggtgagtactcaaccaagtcattctgagaatagtgtatgcggcgaccgagttgctcttgcccggcgtcaatacgggataataccgcgccacatagcagaactttaaaagtgctcatcattggaaaacgttcttcggggcgaaaactctcaaggatcttaccgctgttgagatccagttcgatgtaacccactcgtgcacccaactgatcttcagcatcttttactttcaccagcgtttctgggtgagcaaaaacaggaaggcaaaatgccgcaaaaaagggaataagggcgacacggaaatgttgaatactcatactcttcctttttcaatattattgaagcatttatcagggttattgtctcatgagcggatacatatttgaatgtatttagaaaaataaacaaataggggttccgcgcacatttccccgaaaagtgccacctgacgtctaagaaaccattattatcatgacattaacctataaaaataggcgtatcacgaggccctttcgtc

SEQ ID NO: 21 - DNA, 3831 bp, synthetic construct
  source 1..3831: mol_type = other DNA
ggatccaccatgttcgtgttcctggtgctgctgcctctggtgtccagccagtgcgtgaatctgaccactcggacccagttaccgcctgcttataccaacagcttcaccagaggagtgtactatcctgacaaggtgttcagaagctccgtgctccacagcacacaggacctgtttctgccattcttcagcaatgtgacctggttccacgtgatctccggaaccaacggcacaaagagatttgataaccctgttctgccattcaacgacggcgtgtacttcgcttccatcgagaagtccaacatcatcagaggctggatcttcggcaccaccctggatagcaagacccagagcctcctgatcgtgaacaacgccacgaacgtcgtgatcaaggtgtgcgagttccagttctgtaatgaccccttcttggaccacaagaacaacaagagctggatggaatctgagtttagagtatattccagcgctaacaattgcaccttcgagtacgttagccagcccttcctcatggacctggaaggcaagcagggcaatttcaagaacctgagagagttcgtattcaagaacatcgacggctacttcaagatctacagcaagcacacacctatcatcgtgcgcgagccagaggatctgccacagggcttcagcgctctggaacccctggtcgatctgcctataggcatcaacatcaccagattccaaaccctgctggcgctgcacagatcctacctgacccctggagacagctctagcggatggaccgccggcgctgccgcctactacgtaggctacctgcagcctaggaccttcctgctgaagtacaacgagaacggcaccatcaccgatgccgtggactgtgccctggaccctctatctgagacaaagtgcaccctgaagagcttcaccgtggaaaagggcatctaccagaccagtaactttagagtgcagcccaccgaaagcatcgtgagattccctaacatcaccaatctgtgtcctttcgacgaggtgtttaacgccacaagattcgccagcgtctacgcctggaaccggaagcggatcagcaactgcgtggctgattactccgtcctttataacctggctcccttcttcacatttaaatgctacggagtgagcccaacaaagctgaacgacctgtgcttcaccaacgtgtacgccgatagcttcgtgatcagaggcgatgaggtgagacagattgcccctggccagacaggcaatatcgccgattacaactataagctgcccgacgacttcaccggctgtgtgatcgcttggaacagcaacaagctcgatagcaaggtgagcggaaattacaactacctgtataggctgttcagaaaaagcaatctgaagcctttcgagagagacatcagcaccgaaatctaccaggccggaaataagccttgcaacggcgtggcgggcttcaactgttacttccctctgcgatcatacagcttcagacctacctacggcgtgggccaccagccctaccgagtcgtggtgctgagctttgaactgctgcatgcgcccgcgacagtgtgcggccctaagaaaagcaccaacctggtgaagaacaaatgcgtgaacttcaactttaacgggctgaagggcaccggtgtcctgaccgagagcaacaagaagtttctgcccttccagcaattcggcagagacatcgccgacaccaccgacgccgtccgcgacccccagaccctggagatcctcgatattacaccttgtagcttcggcggcgtcagcgttatcacacccggaacaaacacaagcaatcaggtggccgtgctgtaccagggcgtgaactgcacagaggtgcctgtggcaatccacgccgaccagctgacccctacctggcgggtgtactctaccggcagcaatgtgttccagacaagagccggctgcctgatcggcgccgaatacgtgaacaacagctacgaatgtgacatccctattggcgccggaatctgcgcctcttaccagacacagaccaagtcacatcggagagccagatctgtggcgagccaatctatcatcgcctacaccatgtctctcggcgccgaaaactctgtggcctacagcaacaactctatcgcaatccccacaaacttcaccatcagcgtgacaaccgagatcctgccggtgtctatgaccaagacatccgtggactgcaccatgtacatctgcggcgactccacagaatgcagcaatctgctgttgcagtacggcagcttctgcacacaattaaagcgtgccctgacaggcattgccgtggaacaggataagaatacccaggaagtgttcgcccaggtgaagcagatttacaagaccccacctatcaagtacttcggcggctttaatttctcccagatcctgcctgacccctctaagccttctaagagaagttttatcgaggacctgctgttcaataaagtgaccctggccgatgccgggttcatcaagcagtacggcgattgcctgggcgacatcgccgccagagatcttatttgcgcccagaaattcaagggactgacagtgctgcctcctttgctgaccgacgagatgattgcccagtataccagcgccctgctggccggaaccatcacgtccggctggacattcggcgccggcgccgccttgcagatccccttcgccatgcagatggcctaccggtttaatggcatcggcgtgacgcagaacgtgctgtacgagaaccagaaactgatcgctaaccagtttaactccgccatcggcaagatccaggacagcctgagctccaccgccagcgccctgggcaagctgcaagacgtggtgaaccacaatgcccaagccctgaacaccctggtgaagcagctgagctctaagttcggcgccatcagcagcgtgctgaacgacattttcagcagactggaccctccagaagccgaggtgcagatcgaccggctgatcaccggccggctgcaatccctgcagacctacgtgacccaacagctgatccgggccgccgagatcagagcctcggctaacctggccgccacaaagatgagcgagtgcgtgctgggccagtctaaaagagtggacttctgcggtaaaggataccacctgatgagttttcctcaaagcgcccctcacggcgtggtgttcctgcatgtgacatacgtccccgcccaggagaagaattttaccacagcccctgctatctgtcacgatggcaaagcccacttcccacgggagggcgtgtttgtgagcaacggcacccactggttcgtgacccagagaaacttctacgaacctcagatcatcacgaccgacaacacctttgtgagcggcaactgcgacgtggtgatcggcatcgtgaacaataccgtgtacgaccctctgcagcccgaactggattctttcaaggaggaactggacaagtacttcaagaaccacaccagccctgatgtggacctgggcgacatcagcggcatcaatgcctccgtggtgaatatccagaaagagatcgacagactgaatgaggtggctaagaaccttaatgagagcctgatcgatctgcaggagctgggcaagtacgagcagtacatcaagtggccttggtacatctggctgggattcatcgccggactgatcgctatcgtgatggtcaccatcatgctgtgctgcatgaccagctgctgtagctgcctgaagggatgctgtagctgtggcagctgctgcaagttcgacgaggatgacagcgagcctgtgctgaagggcgtgaagctgcactacacctgataatctaga

SEQ ID NO: 22 - DNA, 3831 bp, synthetic construct
  source 1..3831: mol_type = other DNA
ggatccaccatgttcgtgttcctggtgctgctgcctctggtgtccagccagtgcgtgaatctgaccactcggacccagttaccgcctgcttataccaacagcttcaccagaggagtgtactatcctgacaaggtgttcagaagctccgtgctccacagcacacaggacctgtttctgccattcttcagcaatgtgacctggttccacgtgatctccggaaccaacggcacaaagagatttgataaccctgttctgccattcaacgacggcgtgtacttcgcttccatcgagaagtccaacatcatcagaggctggatcttcggcaccaccctggatagcaagacccagagcctcctgatcgtgaacaacgccacgaacgtcgtgatcaaggtgtgcgagttccagttctgtaatgaccccttcttggaccacaagaacaacaagagctggatggaatctgagtttagagtatattccagcgctaacaattgcaccttcgagtacgttagccagcccttcctcatggacctggaaggcaagcagggcaatttcaagaacctgagagagttcgtattcaagaacatcgacggctacttcaagatctacagcaagcacacacctatcatcgtgcgcgagccagaggatctgccacagggcttcagcgctctggaacccctggtcgatctgcctataggcatcaacatcaccagattccaaaccctgctggcgctgcacagatcctacctgacccctggagacagctctagcggatggaccgccggcgctgccgcctactacgtaggctacctgcagcctaggaccttcctgctgaagtacaacgagaacggcaccatcaccgatgccgtggactgtgccctggaccctctatctgagacaaagtgcaccctgaagagcttcaccgtggaaaagggcatctaccagaccagtaactttagagtgcagcccaccgaaagcatcgtgagattccctaacatcaccaatctgtgtcctttcgacgaggtgtttaacgccacaagattcgccagcgtctacgcctggaaccggaagcggatcagcaactgcgtggctgattactccgtcctttataacctggctcccttcttcacatttaaatgctacggagtgagcccaacaaagctgaacgacctgtgcttcaccaacgtgtacgccgatagcttcgtgatcagaggcgatgaggtgagacagattgcccctggccagacaggcaatatcgccgattacaactataagctgcccgacgacttcaccggctgtgtgatcgcttggaacagcaacaagctcgatagcaaggtgagcggaaattacaactacctgtataggctgttcagaaaaagcaatctgaagcctttcgagagagacatcagcaccgaaatctaccaggccggaaataagccttgcaacggcgtggcgggcttcaactgttacttccctctgcgatcatacagcttcagacctacctacggcgtgggccaccagccctaccgagtcgtggtgctgagctttgaactgctgcatgcgcccgcgacagtgtgcggccctaagaaaagcaccaacctggtgaagaacaaatgcgtgaacttcaactttaacgggctgaagggcaccggtgtcctgaccgagagcaacaagaagtttctgcccttccagcaattcggcagagacatcgccgacaccaccgacgccgtccgcgacccccagaccctggagatcctcgatattacaccttgtagcttcggcggcgtcagcgttatcacacccggaacaaacacaagcaatcaggtggccgtgctgtaccagggcgtgaactgcacagaggtgcctgtggcaatccacgccgaccagctgacccctacctggcgggtgtactctaccggcagcaatgtgttccagacaagagccggctgcctgatcggcgccgaatacgtgaacaacagctacgaatgtgacatccctattggcgccggaatctgcgcctcttaccagacacagaccaagtcacatcggagagccagatctgtggcgagccaatctatcatcgcctacaccatgtctctcggcgccgaaaactctgtggcctacagcaacaactctatcgcaatccccacaaacttcaccatcagcgtgacaaccgagatcctgccggtgtctatgaccaagacatccgtggactgcaccatgtacatctgcggcgactccacagaatgcagcaatctgctgttgcagtacggcagcttctgcacacaattaaagcgtgccctgacaggcattgccgtggaacaggataagaatacccaggaagtgttcgcccaggtgaagcagatttacaagaccccacctatcaagtacttcggcggctttaatttctcccagatcctgcctgacccctctaagccttctaagagaagtcctatcgaggacctgctgttcaataaagtgaccctggccgatgccgggttcatcaagcagtacggcgattgcctgggcgacatcgccgccagagatcttatttgcgcccagaaattcaagggactgacagtgctgcctcctttgctgaccgacgagatgattgcccagtataccagcgccctgctggccggaaccatcacgtccggctggacattcggcgccggccccgccttgcagatccccttccccatgcagatggcctaccggtttaatggcatcggcgtgacgcagaacgtgctgtacgagaaccagaaactgatcgctaaccagtttaactccgccatcggcaagatccaggacagcctgagctccacccctagcgccctgggcaagctgcaagacgtggtgaaccacaatgcccaagccctgaacaccctggtgaagcagctgagctctaagttcggcgccatcagcagcgtgctgaacgacattttcagcagactggaccctccagaagccgaggtgcagatcgaccggctgatcaccggccggctgcaatccctgcagacctacgtgacccaacagctgatccgggccgccgagatcagagcctcggctaacctggccgccacaaagatgagcgagtgcgtgctgggccagtctaaaagagtggacttctgcggtaaaggataccacctgatgagttttcctcaaagcgcccctcacggcgtggtgttcctgcatgtgacatacgtccccgcccaggagaagaattttaccacagcccctgctatctgtcacgatggcaaagcccacttcccacgggagggcgtgtttgtgagcaacggcacccactggttcgtgacccagagaaacttctacgaacctcagatcatcacgaccgacaacacctttgtgagcggcaactgcgacgtggtgatcggcatcgtgaacaataccgtgtacgaccctctgcagcccgaactggattctttcaaggaggaactggacaagtacttcaagaaccacaccagccctgatgtggacctgggcgacatcagcggcatcaatgcctccgtggtgaatatccagaaagagatcgacagactgaatgaggtggctaagaaccttaatgagagcctgatcgatctgcaggagctgggcaagtacgagcagtacatcaagtggccttggtacatctggctgggattcatcgccggactgatcgctatcgtgatggtcaccatcatgctgtgctgcatgaccagctgctgtagctgcctgaagggatgctgtagctgtggcagctgctgcaagttcgacgaggatgacagcgagcctgtgctgaagggcgtgaagctgcactacacctgataatctaga

SEQ ID NO: 23 - DNA, 3840 bp, synthetic construct
  source 1..3840: mol_type = other DNA
ggatccaccatgttcgtgttcctggtgctgctgcctctggtgtccagccagtgcgtgaatctgaccactcggacccagttaccgcctgcttataccaacagcttcaccagaggagtgtactatcctgacaaggtgttcagaagctccgtgctccacagcacacaggacctgtttctgccattcttcagcaatgtgacctggttccacgccatccacgtgtccggaaccaacggcacaaagagatttgataaccctgttctgccattcaacgacggcgtgtacttcgcttccacagagaagtccaacatcatcagaggctggatcttcggcaccaccctggatagcaagacccagagcctcctgatcgtgaacaacgccacgaacgtcgtgatcaaggtgtgcgagttccagttctgtaatgaccccttcttgggcgtttattaccacaagaacaacaagagctggatggaatctgagtttagagtatattccagcgctaacaattgcaccttcgagtacgttagccagcccttcctcatggacctggaaggcaagcagggcaatttcaagaacctgagagagttcgtattcaagaacatcgacggctacttcaagatctacagcaagcacacacctatcaacctagtgcgcgatctgccacagggcttcagcgctctggaacccctggtcgatctgcctataggcatcaacatcaccagattccaaaccctgctggcgctgcacagatcctacctgacccctggagacagctctagcggatggaccgccggcgctgccgcctactacgtaggctacctgcagcctaggaccttcctgctgaagtacaacgagaacggcaccatcaccgatgccgtggactgtgccctggaccctctatctgagacaaagtgcaccctgaagagcttcaccgtggaaaagggcatctaccagaccagtaactttagagtgcagcccaccgaaagcatcgtgagattccctaacatcaccaatctgtgtcctttcggcgaggtgtttaacgccacaagattcgccagcgtctacgcctggaaccggaagcggatcagcaactgcgtggctgattactccgtcctttataacagcgctagcttcagcacatttaaatgctacggagtgagcccaacaaagctgaacgacctgtgcttcaccaacgtgtacgccgatagcttcgtgatcagaggcgatgaggtgagacagattgcccctggccagacaggcaagatcgccgattacaactataagctgcccgacgacttcaccggctgtgtgatcgcttggaacagcaacaacctcgatagcaaggtgggaggaaattacaactacctgtataggctgttcagaaaaagcaatctgaagcctttcgagagagacatcagcaccgaaatctaccaggccggatctacaccttgcaacggcgtggagggcttcaactgttacttccctctgcaatcatacggcttccagcctaccaacggcgtgggctaccagccctaccgagtcgtggtgctgagctttgaactgctgcatgcgcccgcgacagtgtgcggccctaagaaaagcaccaacctggtgaagaacaaatgcgtgaacttcaactttaacgggctgactggcaccggtgtcctgaccgagagcaacaagaagtttctgcccttccagcaattcggcagagacatcgccgacaccaccgacgccgtccgcgacccccagaccctggagatcctcgatattacaccttgtagcttcggcggcgtcagcgttatcacacccggaacaaacacaagcaatcaggtggccgtgctgtaccagggcgtgaactgcacagaggtgcctgtggcaatccacgccgaccagctgacccctacctggcgggtgtactctaccggcagcaatgtgttccagacaagagccggctgcctgatcggcgccgaacacgtgaacaacagctacgaatgtgacatccctattggcgccggaatctgcgcctcttaccagacacagaccaactcacctcggagagccagatctgtggcgagccaatctatcatcgcctacaccatgtctctcggcgccgaaaactctgtggcctacagcaacaactctatcgcaatccccacaaacttcaccatcagcgtgacaaccgagatcctgccggtgtctatgaccaagacatccgtggactgcaccatgtacatctgcggcgactccacagaatgcagcaatctgctgttgcagtacggcagcttctgcacacaattaaatcgtgccctgacaggcattgccgtggaacaggataagaatacccaggaagtgttcgcccaggtgaagcagatttacaagaccccacctatcaaggacttcggcggctttaatttctcccagatcctgcctgacccctctaagccttctaagagaagttttatcgaggacctgctgttcaataaagtgaccctggccgatgccgggttcatcaagcagtacggcgattgcctgggcgacatcgccgccagagatcttatttgcgcccagaaattcaacggactgacagtgctgcctcctttgctgaccgacgagatgattgcccagtataccagcgccctgctggccggaaccatcacgtccggctggacattcggcgccggcgccgccttgcagatccccttcgccatgcagatggcctaccggtttaatggcatcggcgtgacgcagaacgtgctgtacgagaaccagaaactgatcgctaaccagtttaactccgccatcggcaagatccaggacagcctgagctccaccgccagcgccctgggcaagctgcaagacgtggtgaaccagaatgcccaagccctgaacaccctggtgaagcagctgagctctaacttcggcgccatcagcagcgtgctgaacgacattctgagcagactggaccctccagaagccgaggtgcagatcgaccggctgatcaccggccggctgcaatccctgcagacctacgtgacccaacagctgatccgggccgccgagatcagagcctcggctaacctggccgccacaaagatgagcgagtgcgtgctgggccagtctaaaagagtggacttctgcggtaaaggataccacctgatgagttttcctcaaagcgcccctcacggcgtggtgttcctgcatgtgacatacgtccccgcccaggagaagaattttaccacagcccctgctatctgtcacgatggcaaagcccacttcccacgggagggcgtgtttgtgagcaacggcacccactggttcgtgacccagagaaacttctacgaacctcagatcatcacgaccgacaacacctttgtgagcggcaactgcgacgtggtgatcggcatcgtgaacaataccgtgtacgaccctctgcagcccgaactggattctttcaaggaggaactggacaagtacttcaagaaccacaccagccctgatgtggacctgggcgacatcagcggcatcaatgcctccgtggtgaatatccagaaagagatcgacagactgaatgaggtggctaagaaccttaatgagagcctgatcgatctgcaggagctgggcaagtacgagcagtacatcaagtggccttggtacatctggctgggattcatcgccggactgatcgctatcgtgatggtcaccatcatgctgtgctgcatgaccagctgctgtagctgcctgaagggatgctgtagctgtggcagctgctgcaagttcgacgaggatgacagcgagcctgtgctgaagggcgtgaagctgcactacacctgataatctaga